European Patent Application EP 4 534 552 A1, published April 9, 2025. Title: Highly efficient method for obtaining and purification of human Elp123 complex. Applicant: Uniwersytet Jagiellonski. The sequence listing filed with the application follows.

SEQUENCE LISTING (1 sequence)

SEQ ID NO: 1 - DNA, 4776 bp, synthetic construct
  source 1..4776: mol_type = other DNA
gacgcgccctgtagcggcgcattaagcgcggcgggtgtggtggttacgcgcagcgtgaccgctacacttgccagcgccctagcgcccgctcctttcgctttcttcccttcctttctcgccacgttcgccggctttccccgtcaagctctaaatcgggggctccctttagggttccgatttagtgctttacggcacctcgaccccaaaaaacttgattagggtgatggttcacgtagtgggccatcgccctgatagacggtttttcgccctttgacgttggagtccacgttctttaatagtggactcttgttccaaactggaacaacactcaaccctatctcggtctattcttttgatttataagggattttgccgatttcggcctattggttaaaaaatgagctgatttaacaaaaatttaacgcgaattttaacaaaatattaacgtttacaatttcaggtggcacttttcggggaaatgtgcgcggaacccctatttgtttatttttctaaatacattcaaatatgtatccgctcatgagacaataaccctgataaatgcttcaataatattgaaaaaggaagagtatgagtattcaacatttccgtgtcgcccttattcccttttttgcggcattttgccttcctgtttttgctcacccagaaacgctggtgaaagtaaaagatgctgaagatcagttgggtgcacgagtgggttacatcgaactggatctcaacagcggtaagatccttgagagttttcgccccgaagaacgttttccaatgatgagcacttttaaagttctgctatgtggcgcggtattatcccgtattgacgccgggcaagagcaactcggtcgccgcatacactattctcagaatgacttggttgagtactcaccagtcacagaaaagcatcttacggatggcatgacagtaagagaattatgcagtgctgccataaccatgagtgataacactgcggccaacttacttctgacaacgatcggaggaccgaaggagctaaccgcttttttgcacaacatgggggatcatgtaactcgccttgatcgttgggaaccggagctgaatgaagccataccaaacgacgagcgtgacaccacgatgcctgtagcaatggcaacaacgttgcgcaaactattaactggcgaactacttactctagcttcccggcaacaattaatagactggatggaggcggataaagttgcaggaccacttctgcgctcggcccttccggctggctggtttattgctgataaatctggagccggtgagcgtgggtctcgcggtatcattgcagcactggggccagatggtaagccctcccgtatcgtagttatctacacgacggggagtcaggcaactatggatgaacgaaatagacagatcgctgagataggtgcctcactgattaagcattggtaactgtcagaccaagtttactcatatatactttagattgatttaaaacttcatttttaatttaaaaggatctaggtgaagatcctttttgataatctcatgaccaaaatcccttaacgtgagttttcgttccactgagcgtcagaccccgtagaaaagatcaaaggatcttcttgagatcctttttttctgcgcgtaatctgctgcttgcaaacaaaaaaaccaccgctaccagcggtggtttgtttgccggatcaagagctaccaactctttttccgaaggtaactggcttcagcagagcgcagataccaaatactgtccttctagtgtagccgtagttaggccaccacttcaagaactctgtagcaccgcctacatacctcgctctgctaatcctgttaccagtggctgctgccagtggcgataagtcgtgtcttaccgggttggactcaagacgatagttaccggataaggcgcagcggtcgggctgaacggggggttcgtgcacacagcccagcttggagcgaacgacctacaccgaactgagatacctacagcgtgagcattgagaaagcgccacgcttcccgaagggagaaaggcggacaggtatccggtaagcggcagggtcggaacaggagagcgcacgagggagcttccagggggaaacgcctggtatctttatagtcctgtcgggtttcgccacctctgacttgagcgtcgatttttgtgatgctcgtcaggggggcggagcctatggaaaaacgccagcaacgcggcctttttacggttcctggccttttgctggccttttgctcacatgttctttcctgcgttatcccctgattctgtggataaccgtattaccgcctttgagtgagctgataccgctcgccgcagccgaacgaccgagcgcagcgagtcagtgagcgaggaagcggaagagcgcctgatgcggtattttctccttacgcatctgtgcggtatttcacaccgcagaccagccgcgtaacctggcaaaatcggttacggttgagtaataaatggatgccctgcgtaagcgggtgtgggcggacaataaagtcttaaactgaacaaaatagatctaaactatgacaataaagtcttaaactagacagaatagttgtaaactgaaatcagtccagttatgctgtgaaaaagcatactggacttttgttatggctaaagcaaactcttcattttctgaagtgcaaattgcccgtcgtattaaagaggggcgtggccaagggcatggtaaagactatattcgcggcgttgtgacaatttaccgaacaactccgcggccgggaagccgatctcggcttgaacgaattgttaggtggcggtacttgggtcgatatcaaagtgcatcacttcttcccgtatgcccaactttgtatagagagccactgcgggatcgtcaccgtaatctgcttgcacgtagatcacataagcaccaagcgcgttggcctcatgcttgaggagattgatgagcgcggtggcaatgccctgcctccggtgctcgccggagactgcgagatcatagatatagatctcactacgcggctgctcaaacctgggcagaacgtaagccgcgagagcgccaacaaccgcttcttggtcgaaggcagcaagcgcgatgaatgtcttactacggagcaagttcccgaggtaatcggagtccggctgatgttgggagtaggtggctacgtctccgaactcacgaccgaaaagatcaagagcagcccgcatggatttgacttggtcagggccgagcctacatgtgcgaatgatgcccatacttgagccacctaactttgttttagggcgactgccctgctgcgtaacatcgttgctgctgcgtaacatcgttgctgctccataacatcaaacatcgacccacggcgtaacgcgcttgctgcttggatgcccgaggcatagactgtacaaaaaaacagtcataacaagccatgaaaaccgccactgcgccgttaccaccgctgcgttcggtcaaggttctggaccagttgcgtgagcgcatacgctacttgcattacagtttacgaaccgaacaggcttatgtcaactgggttcgtgccttcatccgtttccacggtgtgcgtcacccggcaaccttgggcagcagcgaagtcgaggcatttctgtcctggctggcgaacgagcgcaaggtttcggtctccacgcatcgtcaggcattggcggccttgctgttcttctacggcaaggtgctgtgcacggatctgccctggcttcaggagatcggaagacctcggccgtcgcggcgcttgccggtggtgctgaccccggatgaagtggttcgcatcctcggttttctggaaggcgagcatcgtttgttcgcccaggactctagctatagttctagtggttggctacgtatactccggaatattaatagatcatggagataattaaaatgataaccatctcgcaaataaataagtattttactgttttcgtaacagttttgtaataaaaaaacctataaatattccggattattcataccgtcccaccatcgggcgcggatcccggtccgaagcgcgcggaattcaaaggcctacgtcgacgagctcactagtcgcggccgctttcgaatctagagcctgcagtctcgaggcatgcggtaccaagcttgtcgagaagtactagaggatcataatcagccataccacatttgtagaggttttacttgctttaaaaaacctcccacacctccccctgaacctgaaacataaaatgaatgcaattgttgttgttaacttgtttattgcagcttataatggttacaaataaagcaatagcatcacaaatttcacaaataaagcatttttttcactgcattctagttgtggtttgtccaaactcatcaatgtatcttatcatgtctggatctgatcactgcttgagcctaggagatccgaaccagataagtgaaatctagttccaaactattttgtcatttttaattttcgtattagcttacgacgctacacccagttcccatctattttgtcactcttccctaaataatccttaaaaactccatttccacccctcccagttcccaactattttgtccgcccacagcggggcatttttcttcctgttatgtttttaatcaaacatcctgccaactccatgtgacaaaccgtcatcttcggctactttttctctgtcacagaatgaaaatttttctgtcatctcttcgttattaatgtttgtaattgactgaatatcaacgcttatttgcagcctgaatggcgaatgg